European Patent Application EP 4 553 163 A1, published May 14, 2025. Title: Fatty Acid Synthase. Applicant: Max-Planck-Gesellschaft zur Foerderung der Wissenschaften e.V. Application EP. The sequence listing filed with the application follows.

SEQUENCE LISTING (7 sequences)

SEQ ID NO: 1 - protein, 511 aa, Saccharomyces cerevisiae
KNPNWLEEYHPKLIKNKSGKIFVETKFSKLIGRPPLLVPGMTPCTVSPDFVAATTNAGYTIELAGGGYFSAAGMTAAIDSVVSQIEKGSTFGINLIYVNPFMLQWGIPLIKELRSKGYPIQFLTIGAGVPSLEVASEYIETLGLKYLGLKPGSIDAISQVINIAKAHPNFPIALQWTGGRGGGHHSFEDAHTPMLQMYSKIRRHPNIMLIFGSGFGSADDTYPYLTGEWSTKFDYPPMPFDGFLFGSRVMIAKEVKTSPDAKKCIAACTGVPDDKWEQTYKKPTGGIVTVRSEMGEPIHKIATRGVMLWKEFDETIFNLPKNKLVPTLEAKRDYIISRLNADFQKPWFATVNGQARDLATMTYEEVAKRLVELMFIRSTNSWFDVTWRTFTGDFLRRVEERFTKSKTLSLIQSYSLLDKPDEAIEKVFNAYPAAREQFLNAQDIDHFLSMCQNPMQKPVPFVPVLDRRFEIFFKKDSLWQSEHLEAVVDQDVQRTCILHGPVAAQFTKVID

SEQ ID NO: 2 - protein, 556 aa, Saccharomyces cerevisiae
MDAYSTRPLTLSHGSLEHVLLVPTASFFIASQLQEQFNKILPEPTEGFAADDEPTTPAELVGKFLGYVSSLVEPSKVGQFDQVLNLCLTEFENCYLEGNDIHALAAKLLQENDTTLVKTKELIKNYITARIMAKRPFDKKSNSALFRAVGEGNAQLVAIFGGQGNTDDYFEELRDLYQTYHVLVGDLIKFSAETLSELIRTTLDAEKVFTQGLNILEWLENPSNTPDKDYLLSIPISCPLIGVIQLAHYVVTAKLLGFTPGELRSYLKGATGHSQGLVTAVAIAETDSWESFFVSVRKAITVLFFIGVRCYEAYPNTSLPPSILEDSLENNEGVPSPMLSISNLTQEQVQDYVNKTNSHLPAGKQVEISLVNGAKNLVVSGPPQSLYGLNLTLRKAKAPSGLDQSRIPFSERKLKFSNRFLPVASPFHSHLLVPASDLINKDLVKNNVSFNAKDIQIPVYDTFDGSDLRVLSGSISERIVDCIIRLPVKWETTTQFKATHILDFGPGGASGLGVLTHRNKDGTGVRVIVAGTLDINPDDDYGFKQEIFDVTSNGLK

SEQ ID NO: 3 - protein, 770 aa, Saccharomyces cerevisiae
NSADAAYAQVEIQPRANIQLDFPELKPYKQVKQIAPAELEGLLDLERVIVVTGFAEVGPWGSARTRWEMEAFGEFSLEGCVEMAWIMGFISYHNGNLKGRPYTGWVDSKTKEPVDDKDVKAKYETSILEHSGIRLIEPELFNGYNPEKKEMIQEVIVEEDLEPFEASKETAEQFKHQHGDKVDIFEIPETGEYSVKLLKGATLYIPKALRFDRLVAGQIPTGWNAKTYGISDDIISQVDPITLFVLVSVVEAFIASGITDPYEMYKYVHVSEVGNCSGSGMGGVSALRGMFKDRFKDEPVQNDILQESFINTMSAWVNMLLISSSGPIKTPVGACATSVESVDIGVETILSGKARICIVGGYDDFQEEGSFEFGNMKATSNTLEEFEHGRTPAEMSRPATTTRNGFMEAQGAGIQIIMQADLALKMGVPIYGIVAMAATATDKIGRSVPAPGKGILTTAREHHSSVKYASPNLNMKYRKRQLVTREAQIKDWVENELEALKLEAEEIPSEDQNEFLLERTREIHNEAESQLRAAQQQWGNDFYKRDPRIAPLRGALATYGLTIDDLGVASFHGTSTKANDKNESATINEMMKHLGRSEGNPVIGVFQKFLTGHPKGAAGAWMMNGALQILNSGIIPGNRNADNVDKILEQFEYVLYPSKTLKTDGVRAVSITSFGFGQKGGQAIVVHPDYLYGAITEDRYNEYVAKVSAREKSAYKFFHNGMIYNKLFVSKEHAPYTDELEEDVYLDPLARVSKDKKSGSLTFNSKNIQS

SEQ ID NO: 4 - protein, 417 aa, Saccharomyces cerevisiae
FNPDNGFAPISEVMEDRNQRIKEMYWKLWIDEPFNLDFDPRDVIKGKDFEITAKEVYDFTHAVGNNCEDFVSRPDRTMLAPMDFAIVVGWRAIIKAIFPNTVDGDLLKLVHLSNGYKMIPGAKPLQVGDVVSTTAVIESVVNQPTGKIVDVVGTLSRNGKPVMEVTSSFFYRGNYTDFENTFQKTVEPVYQMHIKTSKDIAVLRSKEWFQLDDEDFDLLNKTLTFETETEVTFKNANIFSSVKCFGPIKVELPTKETVEIGIVDYEAGASHGNPVVDFLKRNGSTLEQKVNLENPIPIAVLDSYTPSTNEPYARVSGDLNPIHVSRHFASYANLPGTITHGMFSSASVRALIENWAADSVSSRVRGYTCQFVDMVLPNTALKTSIQHVGMINGRKLIKFETRNEDDVVVLTGEAEIE

SEQ ID NO: 5 - protein, 643 aa, Saccharomyces cerevisiae
LEEITKDHKVLARQQLQVLARYLKMDLDNGERKFLKEKDTVAELQAQLDYLNAELGEFFVNGVATSFSRKKARTFDSSWNWAKQSLLSLYFEIIHGVLKNVDREVVSEAINIMNRSNDALIKFMEYHISNTDETKGENYQLVKTLGEQLIENCKQVLDVDPVYKDVAKPTGPKTAIDKNGNITYSEEPREKVRKLSQYVQEMALGGPITKESQPTIEEDLTRVYKAISAQADKQDISSSTRVEFEKLYSDLMKFLESSKEIDPSQTTQLAGMDVEDALDKDSTKEVASLPNKSTISKTVSSTIPRETIPFLHLRKKTPAGDWKYDRQLSSLFLDGLEKAAFNGVTFKDKYVLITGAGKGSIGAEVLQGLLQGGAKVVVTTSRFSKQVTDYYQSIYAKYGAKGSTLIVVPFNQGSKQDVEALIEFIYDTEKNGGLGWDLDAIIPFAAIPEQGIELEHIDSKSEFAHRIMLTNILRMMGCVKKQKSARGIETRPAQVILPMSPNHGTFGGDGMYSESKLSLETLFNRWHSESWANQLTVCGAIIGWTRGTGLMSANNIIAEGIEKMGVRTFSQKEMAFNLLGLLTPEVVELCQKSPVMADLNGGLQFVPELKEFTAKLRKELVETSEVRKAVSIETALEHKVVNG

SEQ ID NO: 6 - protein, 487 aa, Saccharomyces cerevisiae
MKPEVEQELAHILLTELLAYQFASPVRWIETQDVFLKDFNTERVVEIGPSPTLAGMAQRTLKNKYESYDAALSLHREILCYSKDAKEIYYTPDPQPVTTFVFTGQGSQEQGMGMDLYKTSKAAQDVWNRADNHFKDTYGFSILDIVINNPVNLTIHFGGEKGKRIRENYSAMIFETIVDGKLKTEKIFKEINEHSTSYTFRSEKGLLSATQFTQPALTLMEKAAFEDLKSKGLIPADATFAGHSLGEYAALASLADVMSIESLVEVVFYRGMTMQVAVPRDELGRSNYGMIAINPGRVAASFSQEALQYVVERVGKRTGWLVEIVNYNVENQQYVAAGDLRALDTVTNVLNFIKLQKIDIIELQKSLSLEEVEGHLFEIIDEASKKSAVKPRPLKLERGFACIPLVGISVPFHSTYLMNGVKPFKSFLKKNIIKENVKVARLAGKYIPNLTAKPFQVTKEYFQDVYDLTGSEPIKEIIDNWEKYEQS

SEQ ID NO: 7 - protein, 169 aa, Saccharomyces cerevisiae
AAEIADEPVKASLLLHVLVAHKLKKSLDSIPMSKTIKDLVGGKSTVQNEILGDLGKEFGTTPEKPEETPLEELAETFQDTFSGALGKQSSSLLSRLISSKMPGGFTITVARKYLQTRWGLPSGRQDGVLLVALSNEPAARLGSEADAKAFLDSMAQKYASIVGVDLSSA